European Patent Application EP 4 711 450 A1, published March 18, 2026. Title: Enzyme agents for carboxy group formation and their applications. Applicant: AMANO ENZYME INC. The sequence listing filed with the application follows.

SEQUENCE LISTING (24 sequences)

SEQ ID NO: 1 - protein, 239 aa, Marasmius fiardii PR-910
DDEVDFSAHAWQAPGPNDSRSPCPGLNTLANHGFLPRNGKNISIPMIIQAGHDGYHFEADILTIAAKVGLLTSPDDQPTTLSLNDLKAHGVLEHDASLSRQDFALGDNVHFNETLFSTLTNSNPGYDVYNITSAGQVQRARLADSVQNNPNITNTDTTLFIRSAESAFYLSAMGDPIKGVAPKNFVQIFFREERMPIEEGWKRSSTPVTADTLVPLINQITAASQPWEPSGKNCPGILP

SEQ ID NO: 2 - protein, 245 aa, Marasmius fiardii PR-910
DDEVDFSAHAWQAPGPNDSRSPCPGLNTLANHGFLPRNGKNISIPMIIQAGHDGYHFEADILTIAAKVGLLTSPDDQPTTLSLNDLKAHGVLEHDASLSRQDFALGDNVHFNETLFSTLTNSNPGYDVYNITSAGQVQRARLADSVQNNPNITNTDTTLFIRSAESAFYLSAMGDPIKGVAPKNFVQIFFREERMPIEEGWKRSSTPVTADTLVPLINQITAASQPWEPSGKNCPGILPHHHHHH

SEQ ID NO: 3 - protein, 263 aa, Marasmius fiardii PR-910
MKLLSSLVFIAVASTALADDEVDFSAHAWQAPGPNDSRSPCPGLNTLANHGFLPRNGKNISIPMIIQAGHDGYHFEADILTIAAKVGLLTSPDDQPTTLSLNDLKAHGVLEHDASLSRQDFALGDNVHFNETLFSTLTNSNPGYDVYNITSAGQVQRARLADSVQNNPNITNTDTTLFIRSAESAFYLSAMGDPIKGVAPKNFVQIFFREERMPIEEGWKRSSTPVTADTLVPLINQITAASQPWEPSGKNCPGILPHHHHHH

SEQ ID NO: 4 - protein, 245 aa, Dendrothele bispora CBS 962.96
KNGSAEIDWDAHQWQAPGPNDLRGPCPGLNTLANHGFLPRDGRNLNMSVIVDAGFDGYHMQPDVLALAVKVAFLTTDDPFSFTLDDIKLHETIEHDASLSREDFALGDNLHFNETIFSTLANSNPGSDFYNTTSAGEVQRLRLADSEARNPNVTNTDKEFFIRSAESGFYLSVMGDPLAGVAPKEFVQIFFREERLPIAEGWHRSETPINSTTLGPLIGKIEAASNWTTSGGCPIIVLGPDFGSF

SEQ ID NO: 5 - protein, 251 aa, Dendrothele bispora CBS 962.96
KNGSAEIDWDAHQWQAPGPNDLRGPCPGLNTLANHGFLPRDGRNLNMSVIVDAGFDGYHMQPDVLALAVKVAFLTTDDPFSFTLDDIKLHETIEHDASLSREDFALGDNLHFNETIFSTLANSNPGSDFYNTTSAGEVQRLRLADSEARNPNVTNTDKEFFIRSAESGFYLSVMGDPLAGVAPKEFVQIFFREERLPIAEGWHRSETPINSTTLGPLIGKIEAASNWTTSGGCPIIVLGPDFGSFHHHHHH

SEQ ID NO: 6 - protein, 273 aa, Dendrothele bispora CBS 962.96
MLSKSLLLSFCTTALLASVASAKNGSAEIDWDAHQWQAPGPNDLRGPCPGLNTLANHGFLPRDGRNLNMSVIVDAGFDGYHMQPDVLALAVKVAFLTTDDPFSFTLDDIKLHETIEHDASLSREDFALGDNLHFNETIFSTLANSNPGSDFYNTTSAGEVQRLRLADSEARNPNVTNTDKEFFIRSAESGFYLSVMGDPLAGVAPKEFVQIFFREERLPIAEGWHRSETPINSTTLGPLIGKIEAASNWTTSGGCPIIVLGPDFGSFHHHHHH

SEQ ID NO: 7 - protein, 239 aa, Mycena venus
STIDNHQWIAPKATDVRSPCPGLNTLANHGYLPRDGRNISIPMMVQAALDGFNVGVDAILQAAKFGLLSTDDLMTLNLDALKLHNLIEHDASLSRNDLAVTGDNLHFNETIFTTLANSNPGVDYYDPTSAGQVQHDRLAISLATNPNITNTAKEFIVRTRESSFYLSVMGNPLTGVAPKQFVNIFFREERLPIAEGWKKSTTVITGEILNPIMDVIIDNSNWTMTQLCEDLVLGPNLTF

SEQ ID NO: 8 - protein, 245 aa, Mycena venus
STIDNHQWIAPKATDVRSPCPGLNTLANHGYLPRDGRNISIPMMVQAALDGFNVGVDAILQAAKFGLLSTDDLMTLNLDALKLHNLIEHDASLSRNDLAVTGDNLHFNETIFTTLANSNPGVDYYDPTSAGQVQHDRLAISLATNPNITNTAKEFIVRTRESSFYLSVMGNPLTGVAPKQFVNIFFREERLPIAEGWKKSTTVITGEILNPIMDVIIDNSNWTMTQLCEDLVLGPNLTFHHHHHH

SEQ ID NO: 9 - protein, 263 aa, Mycena venus
MNLLLVSLFLVAVATAKGSTIDNHQWIAPKATDVRSPCPGLNTLANHGYLPRDGRNISIPMMVQAALDGFNVGVDAILQAAKFGLLSTDDLMTLNLDALKLHNLIEHDASLSRNDLAVTGDNLHFNETIFTTLANSNPGVDYYDPTSAGQVQHDRLAISLATNPNITNTAKEFIVRTRESSFYLSVMGNPLTGVAPKQFVNIFFREERLPIAEGWKKSTTVITGEILNPIMDVIIDNSNWTMTQLCEDLVLGPNLTFHHHHHH

SEQ ID NO: 10 - protein, 243 aa, Armillaria ostoyae
TVDWKLHEWQAPGASDLRGPCPGLNTLANHGFLPRDGKNITIKMVLDAGLEGFNIDPSILILAAKVGLLTTNAPDSFTLDDLKLHGTIEHDASLSRSDFLLGDNLHFNETIYTTLTQSNPGVDYFNATSAGQVQKKRLADDIIANPGIINTIKEFTVRTRESALYLSVMGDPVTGIAPKKFVDIFFREERMPIEEGWTQPSTLITGQTISPIADIIEETSEWVDNGGCPIIRPGPNSDLISCP

SEQ ID NO: 11 - protein, 249 aa, Armillaria ostoyae
TVDWKLHEWQAPGASDLRGPCPGLNTLANHGFLPRDGKNITIKMVLDAGLEGFNIDPSILILAAKVGLLTTNAPDSFTLDDLKLHGTIEHDASLSRSDFLLGDNLHFNETIYTTLTQSNPGVDYFNATSAGQVQKKRLADDIIANPGIINTIKEFTVRTRESALYLSVMGDPVTGIAPKKFVDIFFREERMPIEEGWTQPSTLITGQTISPIADIIEETSEWVDNGGCPIIRPGPNSDLISCPHHHHHH

SEQ ID NO: 12 - protein, 266 aa, Armillaria ostoyae
MYLSLTFVAAFFSAVHATVDWKLHEWQAPGASDLRGPCPGLNTLANHGFLPRDGKNITIKMVLDAGLEGFNIDPSILILAAKVGLLTTNAPDSFTLDDLKLHGTIEHDASLSRSDFLLGDNLHFNETIYTTLTQSNPGVDYFNATSAGQVQKKRLADDIIANPGIINTIKEFTVRTRESALYLSVMGDPVTGIAPKKFVDIFFREERMPIEEGWTQPSTLITGQTISPIADIIEETSEWVDNGGCPIIRPGPNSDLISCPHHHHHH

SEQ ID NO: 13 - DNA, 717 bp, synthetic construct
  source 1..717: mol_type = other DNA
gatgatgaggtggatttcagtgctcacgcttggcaagctccaggcccgaacgatagtcgatccccatgtcctggccttaacacactcgccaatcatggctttctaccacgcaatggcaagaatatctcgattcccatgatcatccaggcaggacatgacgggtatcacttcgaggcagatatcctgactatcgctgcgaaagttgggctcttgacgagtccagacgatcaacctaccacattgtcccttaacgacctgaaagcccatggtgtactggagcatgacgcttcgctaagcagacaggactttgcattaggcgacaacgtgcacttcaacgagactctcttttccacgctgaccaatagcaatccaggttatgacgtgtacaacatcacctcagcaggtcaagtgcaacgtgccaggcttgcggatagcgtccagaacaatccgaacattaccaatacagacacgacgctcttcattcgctctgccgaatcggcgttttacctgtctgcgatgggagatccgataaagggtgtagcacccaagaacttcgtccagatcttctttcgggaagagcgtatgccgattgaggaagggtggaaacggagctcaacccctgttactgccgatacacttgtccccttgatcaaccagataaccgctgcatctcagccctgggaaccctctggaaagaattgccctggaattcttcct

SEQ ID NO: 14 - DNA, 738 bp, synthetic construct
  source 1..738: mol_type = other DNA
gatgatgaggtggatttcagtgctcacgcttggcaagctccaggcccgaacgatagtcgatccccatgtcctggccttaacacactcgccaatcatggctttctaccacgcaatggcaagaatatctcgattcccatgatcatccaggcaggacatgacgggtatcacttcgaggcagatatcctgactatcgctgcgaaagttgggctcttgacgagtccagacgatcaacctaccacattgtcccttaacgacctgaaagcccatggtgtactggagcatgacgcttcgctaagcagacaggactttgcattaggcgacaacgtgcacttcaacgagactctcttttccacgctgaccaatagcaatccaggttatgacgtgtacaacatcacctcagcaggtcaagtgcaacgtgccaggcttgcggatagcgtccagaacaatccgaacattaccaatacagacacgacgctcttcattcgctctgccgaatcggcgttttacctgtctgcgatgggagatccgataaagggtgtagcacccaagaacttcgtccagatcttctttcgggaagagcgtatgccgattgaggaagggtggaaacggagctcaacccctgttactgccgatacacttgtccccttgatcaaccagataaccgctgcatctcagccctgggaaccctctggaaagaattgccctggaattcttcctcaccatcaccatcatcattag

SEQ ID NO: 15 - DNA, 792 bp, synthetic construct
  source 1..792: mol_type = other DNA
atgaagctcttgtcatcgctagtcttcattgccgttgcttccactgcgttagccgatgatgaggtggatttcagtgctcacgcttggcaagctccaggcccgaacgatagtcgatccccatgtcctggccttaacacactcgccaatcatggctttctaccacgcaatggcaagaatatctcgattcccatgatcatccaggcaggacatgacgggtatcacttcgaggcagatatcctgactatcgctgcgaaagttgggctcttgacgagtccagacgatcaacctaccacattgtcccttaacgacctgaaagcccatggtgtactggagcatgacgcttcgctaagcagacaggactttgcattaggcgacaacgtgcacttcaacgagactctcttttccacgctgaccaatagcaatccaggttatgacgtgtacaacatcacctcagcaggtcaagtgcaacgtgccaggcttgcggatagcgtccagaacaatccgaacattaccaatacagacacgacgctcttcattcgctctgccgaatcggcgttttacctgtctgcgatgggagatccgataaagggtgtagcacccaagaacttcgtccagatcttctttcgggaagagcgtatgccgattgaggaagggtggaaacggagctcaacccctgttactgccgatacacttgtccccttgatcaaccagataaccgctgcatctcagccctgggaaccctctggaaagaattgccctggaattcttcctcaccatcaccatcatcattag

SEQ ID NO: 16 - DNA, 735 bp, synthetic construct
  source 1..735: mol_type = other DNA
aagaatggctcggcagagattgattgggatgcacatcagtggcaagcacctggacccaatgacctgagaggaccttgtccagggctcaacacgttggctaatcacggtttccttcctcgtgatggtcgaaacctcaatatgtcggtgattgtggatgccggatttgacggctatcacatgcaaccggatgtactcgctttggcggtcaaagtcgcgttcttgaccactgatgaccccttttccttcacactcgacgatatcaagctccatgagacgatcgagcatgacgcttctctgtcacgggaagactttgcgctaggggataaccttcacttcaacgaaaccatcttctctacactcgccaacagcaatccgggttccgacttctacaacacgacttcagcaggcgaagtacagcgtttacgccttgcggatagtgaagcccgaaacccgaatgtgacgaacacagacaaagagttctttattcgcagtgcggaatccggcttctacctgtcggttatgggcgatccacttgccggagttgctccaaaggagttcgtccagatcttctttcgcgaggagaggcttcccatagctgagggttggcatcggtcagaaacccccataaacagcaccacactgggaccactcattgggaagattgaagcagccagcaattggaccacttctggtggttgcccgatcatcgttttggggcctgactttggcagtttt

SEQ ID NO: 17 - DNA, 756 bp, synthetic construct
  source 1..756: mol_type = other DNA
aagaatggctcggcagagattgattgggatgcacatcagtggcaagcacctggacccaatgacctgagaggaccttgtccagggctcaacacgttggctaatcacggtttccttcctcgtgatggtcgaaacctcaatatgtcggtgattgtggatgccggatttgacggctatcacatgcaaccggatgtactcgctttggcggtcaaagtcgcgttcttgaccactgatgaccccttttccttcacactcgacgatatcaagctccatgagacgatcgagcatgacgcttctctgtcacgggaagactttgcgctaggggataaccttcacttcaacgaaaccatcttctctacactcgccaacagcaatccgggttccgacttctacaacacgacttcagcaggcgaagtacagcgtttacgccttgcggatagtgaagcccgaaacccgaatgtgacgaacacagacaaagagttctttattcgcagtgcggaatccggcttctacctgtcggttatgggcgatccacttgccggagttgctccaaaggagttcgtccagatcttctttcgcgaggagaggcttcccatagctgagggttggcatcggtcagaaacccccataaacagcaccacactgggaccactcattgggaagattgaagcagccagcaattggaccacttctggtggttgcccgatcatcgttttggggcctgactttggcagttttcaccatcaccatcatcattag

SEQ ID NO: 18 - DNA, 822 bp, synthetic construct
  source 1..822: mol_type = other DNA
atgctgtcgaaatccctgctactatccttctgcaccactgccttgttagcctctgtcgctagcgctaagaatggctcggcagagattgattgggatgcacatcagtggcaagcacctggacccaatgacctgagaggaccttgtccagggctcaacacgttggctaatcacggtttccttcctcgtgatggtcgaaacctcaatatgtcggtgattgtggatgccggatttgacggctatcacatgcaaccggatgtactcgctttggcggtcaaagtcgcgttcttgaccactgatgaccccttttccttcacactcgacgatatcaagctccatgagacgatcgagcatgacgcttctctgtcacgggaagactttgcgctaggggataaccttcacttcaacgaaaccatcttctctacactcgccaacagcaatccgggttccgacttctacaacacgacttcagcaggcgaagtacagcgtttacgccttgcggatagtgaagcccgaaacccgaatgtgacgaacacagacaaagagttctttattcgcagtgcggaatccggcttctacctgtcggttatgggcgatccacttgccggagttgctccaaaggagttcgtccagatcttctttcgcgaggagaggcttcccatagctgagggttggcatcggtcagaaacccccataaacagcaccacactgggaccactcattgggaagattgaagcagccagcaattggaccacttctggtggttgcccgatcatcgttttggggcctgactttggcagttttcaccatcaccatcatcattag

SEQ ID NO: 19 - DNA, 717 bp, synthetic construct
  source 1..717: mol_type = other DNA
tctacgattgacaatcaccagtggattgcacctaaagcgacggatgtccggtcaccatgtcctgggctgaatacacttgcaaaccatggctatctgcctagggatggccgcaacatcagtataccgatgatggtccaagctgccttagacgggttcaatgtaggtgtcgatgcgattctacaagccgctaagtttggccttctaagcactgatgatctcatgacccttaacttggatgccttgaagttacacaacctgatcgagcatgatgccagtttgtcccgtaacgacttggcagtgacaggagacaaccttcacttcaacgagacaatcttcacgacacttgcgaattccaatccaggtgttgactactatgaccccacttcagctggacaagtgcagcatgatcgactcgcaattagcttggcaaccaatcccaacataaccaataccgccaaggagttcatcgtcagaacgcgggaatcttcgttctacctctcggttatgggcaatccgcttactggtgttgctccgaaacagttcgtgaacatcttctttcgcgaagaacgtctgccaattgctgaagggtggaagaagagcactaccgtcattacgggagagatcctgaatcccataatggacgtcatcatcgacaactctaactggaccatgactcagctatgcgaggatctcgtgctcggtcctaatctcaccttt

SEQ ID NO: 20 - DNA, 738 bp, synthetic construct
  source 1..738: mol_type = other DNA
tctacgattgacaatcaccagtggattgcacctaaagcgacggatgtccggtcaccatgtcctgggctgaatacacttgcaaaccatggctatctgcctagggatggccgcaacatcagtataccgatgatggtccaagctgccttagacgggttcaatgtaggtgtcgatgcgattctacaagccgctaagtttggccttctaagcactgatgatctcatgacccttaacttggatgccttgaagttacacaacctgatcgagcatgatgccagtttgtcccgtaacgacttggcagtgacaggagacaaccttcacttcaacgagacaatcttcacgacacttgcgaattccaatccaggtgttgactactatgaccccacttcagctggacaagtgcagcatgatcgactcgcaattagcttggcaaccaatcccaacataaccaataccgccaaggagttcatcgtcagaacgcgggaatcttcgttctacctctcggttatgggcaatccgcttactggtgttgctccgaaacagttcgtgaacatcttctttcgcgaagaacgtctgccaattgctgaagggtggaagaagagcactaccgtcattacgggagagatcctgaatcccataatggacgtcatcatcgacaactctaactggaccatgactcagctatgcgaggatctcgtgctcggtcctaatctcacctttcaccatcaccatcatcattag

SEQ ID NO: 21 - DNA, 792 bp, synthetic construct
  source 1..792: mol_type = other DNA
atgaacctgctcttggtgtccctatttctggtagctgttgccacagcgaaaggctctacgattgacaatcaccagtggattgcacctaaagcgacggatgtccggtcaccatgtcctgggctgaatacacttgcaaaccatggctatctgcctagggatggccgcaacatcagtataccgatgatggtccaagctgccttagacgggttcaatgtaggtgtcgatgcgattctacaagccgctaagtttggccttctaagcactgatgatctcatgacccttaacttggatgccttgaagttacacaacctgatcgagcatgatgccagtttgtcccgtaacgacttggcagtgacaggagacaaccttcacttcaacgagacaatcttcacgacacttgcgaattccaatccaggtgttgactactatgaccccacttcagctggacaagtgcagcatgatcgactcgcaattagcttggcaaccaatcccaacataaccaataccgccaaggagttcatcgtcagaacgcgggaatcttcgttctacctctcggttatgggcaatccgcttactggtgttgctccgaaacagttcgtgaacatcttctttcgcgaagaacgtctgccaattgctgaagggtggaagaagagcactaccgtcattacgggagagatcctgaatcccataatggacgtcatcatcgacaactctaactggaccatgactcagctatgcgaggatctcgtgctcggtcctaatctcacctttcaccatcaccatcatcattag

SEQ ID NO: 22 - DNA, 729 bp, synthetic construct
  source 1..729: mol_type = other DNA
actgtcgattggaaacttcacgaatggcaagctccaggagcatcggacttacgtggtccttgtccgggattgaacactttggccaatcacggctttctacccagagacggaaagaacattacgatcaagatggtgcttgatgccggtctagagggattcaacatagatccctccatcctgattttggctgccaaagtcggcttactcaccacaaatgcaccagacagctttacgcttgatgacctgaagctgcatgggaccattgagcatgatgcgtctttgtcacgctctgatttcctcctcggtgataacttgcacttcaatgagacgatctacaccacccttacgcagtccaatcctggtgtggactacttcaacgcgacatctgctggccaagtccagaaaaaacggcttgcggatgacatcattgccaacccagggatcatcaacaccattaaggagttcacagttcgaacgcgggaaagtgccctctatctctccgtaatgggcgatccagttactggcattgctcccaagaagttcgtggacatattctttcgcgaagagaggatgcctattgaagagggatggactcaaccgagtaccctaatcacagggcagacaatctcgcctatagctgacatcatcgaggaaacttcggaatgggtcgataatggtggctgcccgattatccgtcctggtccgaatagcgacctgatcagctgcccc

SEQ ID NO: 23 - DNA, 750 bp, synthetic construct
  source 1..750: mol_type = other DNA
actgtcgattggaaacttcacgaatggcaagctccaggagcatcggacttacgtggtccttgtccgggattgaacactttggccaatcacggctttctacccagagacggaaagaacattacgatcaagatggtgcttgatgccggtctagagggattcaacatagatccctccatcctgattttggctgccaaagtcggcttactcaccacaaatgcaccagacagctttacgcttgatgacctgaagctgcatgggaccattgagcatgatgcgtctttgtcacgctctgatttcctcctcggtgataacttgcacttcaatgagacgatctacaccacccttacgcagtccaatcctggtgtggactacttcaacgcgacatctgctggccaagtccagaaaaaacggcttgcggatgacatcattgccaacccagggatcatcaacaccattaaggagttcacagttcgaacgcgggaaagtgccctctatctctccgtaatgggcgatccagttactggcattgctcccaagaagttcgtggacatattctttcgcgaagagaggatgcctattgaagagggatggactcaaccgagtaccctaatcacagggcagacaatctcgcctatagctgacatcatcgaggaaacttcggaatgggtcgataatggtggctgcccgattatccgtcctggtccgaatagcgacctgatcagctgcccccaccatcaccatcatcattag

SEQ ID NO: 24 - DNA, 801 bp, synthetic construct
  source 1..801: mol_type = other DNA
atgtatctctcactgacctttgtagcagccttcttttccgcggttcatgcaactgtcgattggaaacttcacgaatggcaagctccaggagcatcggacttacgtggtccttgtccgggattgaacactttggccaatcacggctttctacccagagacggaaagaacattacgatcaagatggtgcttgatgccggtctagagggattcaacatagatccctccatcctgattttggctgccaaagtcggcttactcaccacaaatgcaccagacagctttacgcttgatgacctgaagctgcatgggaccattgagcatgatgcgtctttgtcacgctctgatttcctcctcggtgataacttgcacttcaatgagacgatctacaccacccttacgcagtccaatcctggtgtggactacttcaacgcgacatctgctggccaagtccagaaaaaacggcttgcggatgacatcattgccaacccagggatcatcaacaccattaaggagttcacagttcgaacgcgggaaagtgccctctatctctccgtaatgggcgatccagttactggcattgctcccaagaagttcgtggacatattctttcgcgaagagaggatgcctattgaagagggatggactcaaccgagtaccctaatcacagggcagacaatctcgcctatagctgacatcatcgaggaaacttcggaatgggtcgataatggtggctgcccgattatccgtcctggtccgaatagcgacctgatcagctgcccccaccatcaccatcatcattag